European Patent Specification EP 3 967 649 B1, published November 12, 2025. Title: Lipid nanoparticle. Applicant: Hokkaido University. The sequence listing filed with the application follows.

SEQUENCE LISTING (13 sequences)

SEQ ID NO: 1 - DNA, 20 bp, Aequorea coerulescens
  partial of GFP gene
acggcgtgcagtgcttcagc

SEQ ID NO: 2 - RNA, 36 nt, Artificial Sequence
  Description of Artificial Sequence: Synthesized crRNA
gcugaagcacugcacgccguguuuuagagcuaugcu

SEQ ID NO: 3 - RNA, 67 nt, Artificial Sequence
  Description of Artificial Sequence: Synthesized tracrRNA
agcauagcaaguuaaaauaaggcuaguccguuaucaacuugaaaaaguggcaccgagucggugcuuu

SEQ ID NO: 4 - DNA, 617 bp, Artificial Sequence
  Description of Artificial Sequence: Synthesized dsDNA
tgcccatcctggtcgagctggacggcgacgtaaacggccacaagttcagcgtgtccggcgagggcgagggcgatgccacctacggcaagctgaccctgaagttcatctgcaccaccggcaagctgcccgtgccctggcccaccctcgtgaccaccctgacctacggcgtgcagtgcttcagccgctaccccgaccacatgaagcagcacgacttcttcaagtccgccatgcccgaaggctacgtccaggagcgcaccatcttcttcaaggacgacggcaactacaagacccgcgccgaggtgaagttcgagggcgacaccctggtgaaccgcatcgagctgaagggcatcgacttcaaggaggacggcaacatcctggggcacaagctggagtacaactacaacagccacaacgtctatatcatggccgacaagcagaagaacggcatcaaggtgaacttcaagatccgccacaacatcgaggacggcagcgtgcagctcgccgaccactaccagcagaacacccccatcggcgacggccccgtgctgctgcccgacaaccactacctgagcacccagtccgccctgagcaaagaccccaacgagaagcgcgatcac

SEQ ID NO: 5 - DNA, 132 bp, Artificial Sequence
  Description of Artificial Sequence: Synthesized ssODN for GFP knock out
ctgaagttcatctgcaccaccggcaagctgcccgtgccctggcccaccctcgtgaccaccctgacctacggcgtgcagtgcttcagccgctaccccgaccacatgaagcagcacgacttcttcaagtccgcc

SEQ ID NO: 6 - DNA, 132 bp, Artificial Sequence
  Description of Artificial Sequence: Synthesized ssODN for BFP knock in
ctgaagttcatctgcaccaccggcaagctgcccgtgccctggcccaccctcgtgaccaccctgagccacggggtgcagtgcttcagccgctaccccgaccacatgaagcagcacgacttcttcaagtccgcc

SEQ ID NO: 7 - RNA, 60 nt, Artificial Sequence
  Description of Artificial Sequence: Synthesized ssODN for GFP knock out
ccucgugaccacccugaccuacggcgugcagugcuucagccgcuaccccgaccacaugaa

SEQ ID NO: 8 - RNA, 41 nt, Artificial Sequence
  Description of Artificial Sequence: Synthesized gRNA
uaauuucuacucuuguagaucgucgccguccagcucgacca

SEQ ID NO: 9 - RNA, 100 nt, Artificial Sequence
  Description of Artificial Sequence: Synthesized gRNA
cgaucgcucgguuaggagagaccccagacgcuccggccauacgcgaguccaccaugaauuaauuucuacucuuguagaucgucgccguccagcucgacca

SEQ ID NO: 10 - RNA, 120 nt, Artificial Sequence
  Description of Artificial Sequence: Synthesized ssODN
auggugagcaagggcgaggagcuguucaccgggguggugcccauccuggucgagcuggacggcgacguaaacggccacaaguucagcguguccggcgagggcgagggcgagggcgaugcc

SEQ ID NO: 11 - RNA, 60 nt, Artificial Sequence
  Description of Artificial Sequence: Synthesized ssODN
caccgggguggugcccauccuggucgagcuggacggcgacguaaacggccacaaguucag

SEQ ID NO: 12 - RNA, 36 nt, Artificial Sequence
  Description of Artificial Sequence: Synthesized crRNA
gggcacgggcagcuugccggguuuuagagcuaugcu

SEQ ID NO: 13 - RNA, 36 nt, Artificial Sequence
  Description of Artificial Sequence: Synthesized crRNA
cucgugaccacccugaccuaguuuuagagcuaugcu